European Patent Application EP 4 349 845 A1, published April 10, 2024. Title: New isoflavone compound. Applicant: NABOCUL Cosmetics Co., Ltd. The sequence listing filed with the application follows.

SEQUENCE LISTING (4 sequences)

SEQ ID NO: 1 - DNA, 20 bp, Artificial Sequence
  AQP3 forward primer
agacagccccttcaggattt

SEQ ID NO: 2 - DNA, 20 bp, Artificial Sequence
  AQP3 reverse primer
tcccttgccctgaatatctg

SEQ ID NO: 3 - DNA, 21 bp, Artificial Sequence
  FLG2 forward primer
ctgtggtcattcatggagtgg

SEQ ID NO: 4 - DNA, 22 bp, Artificial Sequence
  FLG2 reverse primer
ccctagaagggctaatgtgtga